European Patent Application EP 4 112 719 A1, published January 4, 2023. Title: 遺伝子ノックイン方法、遺伝子ノックイン細胞作製方法、遺伝子ノックイン細胞、がん化リスク評価方法、がん細胞製造方法、及びこれらに用いるためのキット. Applicant: IMRA JAPAN KABUSHIKIKAISHA. The sequence listing filed with the application follows.

SEQUENCE LISTING (17 sequences)

SEQ ID NO: 1 - DNA, 4152 bp, Artificial Sequence
  MSpCas9
gacaagaagtacagcatcggcctggacatcggcaccaactctgtgggctgggccgtgatcaccgacgagtacaaggtgcccagcaagaaattcaaggtgctgggcaacaccgaccggcacagcatcaagaagaacctgatcggagccctgctgttcgacagcggcgaaacagccgaggccacccggctgaagagaaccgccagaagaagatacaccagacggaagaaccggatctgctatctgcaagagatcttcagcaacgagatggccaaggtggacgacagcttcttccacagactggaagagtccttcctggtggaagaggataagaagcacgagcggcaccccatcttcggcaacatcgtggacgaggtggcctaccacgagaagtaccccaccatctaccacctgagaaagaaactggtggacagcaccgacaaggccgacctgcggctgatctatctggccctggcccacatgatcaagttccggggccacttcctgatcgagggcgacctgaaccccgacaacagcgacgtggacaagctgttcatccagctggtgcagacctacaaccagctgttcgaggaaaaccccatcaacgccagcggcgtggacgccaaggccatcctgtctgccagactgagcaagagcagacggctggaaaatctgatcgcccagctgcccggcgagaagaagaatggcctgttcggaaacctgattgccctgagcctgggcctgacccccaacttcaagagcaacttcgacctggccgaggatgccaaactgcagctgagcaaggacacctacgacgacgacctggacaacctgctggcccagatcggcgaccagtacgccgacctgtttctggccgccaagaacctgtccgacgccatcctgctgagcgacatcctgagagtgaacaccgagatcaccaaggcccccctgagcgcctctatgatcaagagatacgacgagcaccaccaggacctgaccctgctgaaagctctcgtgcggcagcagctgcctgagaagtacaaagagattttcttcgaccagagcaagaacggctacgccggctacattgacggcggagccagccaggaagagttctacaagttcatcaagcccatcctggaaaagatggacggcaccgaggaactgctcgtgaagctgaacagagaggacctgctgcggaagcagcggaccttcgacaacggcagcatcccccaccagatccacctgggagagctgcacgccattctgcggcggcaggaagatttttacccattcctgaaggacaaccgggaaaagatcgagaagatcctgaccttccgcatcccctactacgtgggccctctggccaggggaaacagcagattcgcctggatgaccagaaagagcgaggaaaccatcaccccctggaacttcgaggaagtggtggacaagggcgcttccgcccagagcttcatcgagcggatgaccaacttcgataagaacctgcccaacgagaaggtgctgcccaagcacagcctgctgtacgagtacttcaccgtgtataacgagctgaccaaagtgaaatacgtgaccgagggaatgagaaagcccgccttcctgagcggcgagcagaaaaaggccatcgtggacctgctgttcaagaccaaccggaaagtgaccgtgaagcagctgaaagaggactacttcaagaaaatcgagtgcttcgactccgtggaaatctccggcgtggaagatcggttcaacgcctccctgggcacataccacgatctgctgaaaattatcaaggacaaggacttcctggacaatgaggaaaacgaggacattctggaagatatcgtgctgaccctgacactgtttgaggacagagagatgatcgaggaacggctgaaaacctatgcccacctgttcgacgacaaagtgatgaagcagctgaagcggcggagatacaccggctggggcaggctgagccggaagctgatcaacggcatccgggacaagcagtccggcaagacaatcctggatttcctgaagtccgacggcttcgccaacagagccttcgcggcgctgatcgccgacgacagcctgacctttaaagaggacatccagaaagcccaggtgtccggccagggcgatagcctgcacgagcacattgccaatctggccggcagccccgccattaagaagggcatcctgcagacagtgaaggtggtggacgagctcgtgaaagtgatgggccggcacaagcccgagaacatcgtgatcgaaatggccagagagaaccagaccacccagaagggacagaagaacagccgcgagagaatgaagcggatcgaagagggcatcaaagagctgggcagccagatcctgaaagaacaccccgtggaaaacacccagctgcagaacgagaagctgtacctgtactacctgcagaatgggcgggatatgtacgtggaccaggaactggacatcaaccggctgtccgactacgatgtggaccatatcgtgcctcagagctttctgaaggacgactccatcgacaacaaggtgctgaccagaagcgacaagaaccggggcaagagcgacaacgtgccctccgaagaggtcgtgaagaagatgaagaactactggcggcagctgctgaacgccaagctgattacccagagaaagttcgacaatctgaccaaggccgagagaggcggcctgagcgaactggataaggccggcttcatcaagagacagctggtggaaacccggcagatcacaaagcacgtggcacagatcctggactcccggatgaacactaagtacgacgagaatgacaagctgatccgggaagtgaaagtgatcaccctgaagtccaagctggtgtccgatttccggaaggatttccagttttacaaagtgcgcgagatcaacaactaccaccacgcccacgacgcctacctgaacgccgtcgtgggaaccgccctgatcaaaaagtaccctaagctggaaagcgagttcgtgtacggcgactacaaggtgtacgacgtgcggaagatgatcgccaagagcgagcaggaaatcggcaaggctaccgccaagtacttcttctacagcaacatcatgaactttttcaagaccgagattaccctggccaacggcgagatccggaagcggcctctgatcgagacaaacggcgaaaccggggagatcgtgtgggataagggccgggattttgccaccgtgcggaaagtgctgagcatgccccaagtgaatatcgtgaaaaagaccgaggtgcagacaggcggcttcagcaaagagtctatcctgcccaagaggaacagcgataagctgatcgccagaaagaaggactgggaccctaagaagtacggcggcttcgacagccccaccgtggcctattctgtgctggtggtggccaaagtggaaaagggcaagtccaagaaactgaagagtgtgaaagagctgctggggatcaccatcatggaaagaagcagcttcgagaagaatcccatcgactttctggaagccaagggctacaaagaagtgaaaaaggacctgatcatcaagctgcctaagtactccctgttcgagctggaaaacggccggaagagaatgctggcctctgccggcgaactgcagaagggaaacgaactggccctgccctccaaatatgtgaacttcctgtacctggccagccactatgagaagctgaagggctcccccgaggataatgagcagaaacagctgtttgtggaacagcacaagcactacctggacgagatcatcgagcagatcagcgagttctccaagagagtgatcctggccgacgctaatctggacaaagtgctgtccgcctacaacaagcaccgggataagcccatcagagagcaggccgagaatatcatccacctgtttaccctgaccaatctgggagcccctgccgccttcaagtactttgacaccaccatcgaccggaagaggtacaccagcaccaaagaggtgctggacgccaccctgatccaccagagcatcaccggcctgtacgagacacggatcgacctgtctcagctgggaggcgacaaaaggccggcggccacgaaaaaggccggccaggcaaaaaagaaaaagtaa

SEQ ID NO: 2 - DNA, 21 bp, Artificial Sequence
  MSpCas9 Forward primer
gccttcgcggcgctgatcgcc

SEQ ID NO: 3 - DNA, 20 bp, Artificial Sequence
  MSpCas9 Reverse primer
ccgacggcttcgccaacaga

SEQ ID NO: 4 - DNA, 25 bp, Artificial Sequence
  sgRNA1
caccgcagcagcaacagcacggaaa

SEQ ID NO: 5 - DNA, 25 bp, Artificial Sequence
  sgRNA2
caccgctctctgaacccgcccattg

SEQ ID NO: 6 - DNA, 25 bp, Artificial Sequence
  sgRNA3
aaactttccgtgctgttgctgctgc

SEQ ID NO: 7 - DNA, 25 bp, Artificial Sequence
  sgRNA6
aaaccaatgggcgggttcagagagc

SEQ ID NO: 8 - DNA, 43 bp, Artificial Sequence
  donor hSP3pro Forward primer
cagcagcaacagcacggaaacggcagcagcagcaacagcacgg

SEQ ID NO: 9 - DNA, 43 bp, Artificial Sequence
  donor hSP3pro Reverse primer
ccccaatgggcgggttcagagaggctgagtgtcctacccccaa

SEQ ID NO: 10 - DNA, 20 bp, Artificial Sequence
  hSP3pro Forward primer
tgtgcctgcagctcccgaaa

SEQ ID NO: 11 - DNA, 20 bp, Artificial Sequence
  hSP3pro Reverse primer
ggtagcggccagcagagcga

SEQ ID NO: 12 - DNA, 20 bp, Artificial Sequence
  GAPDH Forward primer
accacagtccatgccatcac

SEQ ID NO: 13 - DNA, 20 bp, Artificial Sequence
  GAPDH Reverse primer
tccaccaccctgttgctgta

SEQ ID NO: 14 - DNA, 20 bp, Artificial Sequence
  hSP3 Forward primer
ccaggatgtggtaaagtcta

SEQ ID NO: 15 - DNA, 20 bp, Artificial Sequence
  hSP3 Reverse primer
ctccattgtctcatttccag

SEQ ID NO: 16 - DNA, 20 bp, Artificial Sequence
  hSP3pro Forward primer 2
cagcagcagcaacagcacgg

SEQ ID NO: 17 - DNA, 20 bp, Artificial Sequence
  hSP3pro Reverse primer 2
gctgagtgtcctacccccaa